European Patent Specification EP 3 606 955 B1, published November 6, 2024. Title: Bispecific Antibodies specifically binding to PD1 and LAG3. Applicant: F. Hoffmann-La Roche AG. The sequence listing filed with the application follows.

SEQUENCE LISTING (169 sequences)

SEQ ID NO: 1 - protein, 7 aa, Artificial Sequence
  heavy chain HVR-H1, PD1-0103
GFSFSSY

SEQ ID NO: 2 - protein, 3 aa, Artificial Sequence
  heavy chain HVR-H2, PD1-0103
GGR

SEQ ID NO: 3 - protein, 9 aa, Artificial Sequence
  heavy chain HVR-H3, PD1-0103
TGRVYFALD

SEQ ID NO: 4 - protein, 11 aa, Artificial Sequence
  light chain HVR-L1, PD1-0103
SESVDTSDNSF

SEQ ID NO: 5 - protein, 3 aa, Artificial Sequence
  light chain HVR-L2, PD1-0103
RSS

SEQ ID NO: 6 - protein, 6 aa, Artificial Sequence
  light chain HVR-L3, PD1-0103
NYDVPW

SEQ ID NO: 7 - protein, 120 aa, Artificial Sequence
  heavy chain variable domain VH, PD1-0103
EVILVESGGGLVKPGGSLKLSCAASGFSFSSYTMSWVRQTPEKRLDWVATISGGGRDIYYPDSVKGRFTISRDNAKNTLYLEMSSLMSEDTALYYCVLLTGRVYFALDSWGQGTSVTVSS

SEQ ID NO: 8 - protein, 111 aa, Artificial Sequence
  light chain variable domain VL, PD1-0103
KIVLTQSPASLPVSLGQRATISCRASESVDTSDNSFIHWYQQRPGQSPKLLIYRSSTLESGVPARFSGSGSRTDFTLTIDPVEADDVATYYCQQNYDVPWTFGGGTKLEIK

SEQ ID NO: 9 - protein, 120 aa, Artificial Sequence
  humanized variant -heavy chain variable domain VH of PD1-0103_01 (PD1 0376)
EVQLLESGGGLVQPGGSLRLSCAASGFSFSSYTMSWVRQAPGKGLEWVATISGGGRDIYYPDSVKGRFTISRDNSKNTLYLQMNSLRAEDTAVYYCVLLTGRVYFALDSWGQGTLVTVSS

SEQ ID NO: 10 - protein, 111 aa, Artificial Sequence
  humanized variant -light chain variable domain VL of PD1-0103_01 (PD1 0376)
DIVMTQSPDSLAVSLGERATINCKASESVDTSDNSFIHWYQQKPGQSPKLLIYRSSTLESGVPDRFSGSGSGTDFTLTISSLQAEDVAVYYCQQNYDVPWTFGQGTKVEIK

SEQ ID NO: 11 - protein, 111 aa, Artificial Sequence
  humanized variant -light chain variable domain VL of PD1-0103_02
DVVMTQSPLSLPVTLGQPASISCRASESVDTSDNSFIHWYQQRPGQSPRLLIYRSSTLESGVPDRFSGSGSGTDFTLKISRVEAEDVGVYYCQQNYDVPWTFGQGTKVEIK

SEQ ID NO: 12 - protein, 111 aa, Artificial Sequence
  humanized variant -light chain variable domain VL of PD1-0103_03
EIVLTQSPATLSLSPGERATLSCRASESVDTSDNSFIHWYQQKPGQSPRLLIYRSSTLESGIPARFSGSGSGTDFTLTISSLEPEDFAVYYCQQNYDVPWTFGQGTKVEIK

SEQ ID NO: 13 - protein, 111 aa, Artificial Sequence; identical to SEQ ID NO: 12
  humanized variant -light chain variable domain VL of PD1-0103_04

SEQ ID NO: 14 - protein, 5 aa, Artificial Sequence
  heavy chain HVR-H1, aLAG3(0414)
DYTMN

SEQ ID NO: 15 - protein, 17 aa, Artificial Sequence
  heavy chain HVR-H2, aLAG3(0414)
VISWDGGGTYYTDSVKG

SEQ ID NO: 16 - protein, 12 aa, Artificial Sequence
  heavy chain HVR-H3, aLAG3(0414)
GLTDTTLYGSDY

SEQ ID NO: 17 - protein, 11 aa, Artificial Sequence
  light chain HVR-L1, aLAG3(0414)
RASQSISSYLN

SEQ ID NO: 18 - protein, 7 aa, Artificial Sequence
  light chain HVR-L2, aLAG3(0414)
AASTLQS

SEQ ID NO: 19 - protein, 9 aa, Artificial Sequence
  light chain HVR-L3, aLAG3(0414)
QQTYSSPLT

SEQ ID NO: 20 - protein, 121 aa, Artificial Sequence
  heavy chain variable domain VH, aLAG3(0414)
EVQLLESGGGLVQPGGSLRLSCAASGFIFDDYTMNWVRQAPGKGLEWVAVISWDGGGTYYTDSVKGRFTISRDDFKNTLYLQMNSLRAEDTAVYYCAKGLTDTTLYGSDYWGQGTLVTVSS

SEQ ID NO: 21 - protein, 107 aa, Artificial Sequence
  light chain variable domain VL, aLAG3(0414)
DIQMTQSPSSLSASVGDRVTITCRASQSISSYLNWYQQKPGKAPKLLIYAASTLQSGVPSRFSGSGSGTDFTLTISSLQPEDFATYYCQQTYSSPLTFGGGTKVEIK

SEQ ID NO: 22 - protein, 5 aa, Artificial Sequence
  heavy chain HVR-H1, aLAG3(0403)
DYTMH

SEQ ID NO: 23 - protein, 17 aa, Artificial Sequence
  heavy chain HVR-H2, aLAG3(0403)
LVSWDGGGTYYTNSVKG

SEQ ID NO: 24 - protein, 12 aa, Artificial Sequence
  heavy chain HVR-H3, aLAG3(0403)
AITDTSLYGYDY

SEQ ID NO: 25 - protein, 11 aa, Artificial Sequence
  light chain HVR-L1, aLAG3(0403)
RASQSISSYLN

SEQ ID NO: 26 - protein, 7 aa, Artificial Sequence
  light chain HVR-L2, aLAG3(0403)
AASSLQS

SEQ ID NO: 27 - protein, 9 aa, Artificial Sequence
  light chain HVR-L3, aLAG3(0403)
QQTYSTPLT

SEQ ID NO: 28 - protein, 121 aa, Artificial Sequence
  heavy chain variable domain VH, aLAG3(0403)
EVQLLESGGGLVQPGGSLRLSCAASGFTFDDYTMHWVRQAPGKGLEWVSLVSWDGGGTYYTNSVKGRFTISRDNSKNTLYLQMNSLRAEDTAVYFCAKAITDTSLYGYDYWGQGILVTVSS

SEQ ID NO: 29 - protein, 107 aa, Artificial Sequence
  light chain variable domain VL, aLAG3(0403)
DIQMTQSPSSLSASVGDRVTITCRASQSISSYLNWYQQKPGNAPKLLIYAASSLQSGVPSRFSGSGSGTDFTLTISSLQPEDFATYYCQQTYSTPLTFGGGTKVEIK

SEQ ID NO: 30 - protein, 5 aa, Artificial Sequence
  heavy chain HVR-H1, aLAG3(0411)
DYTMN

SEQ ID NO: 31 - protein, 17 aa, Artificial Sequence
  heavy chain HVR-H2, aLAG3(0411)
VISWDGGATYYADSVKG

SEQ ID NO: 32 - protein, 12 aa, Artificial Sequence
  heavy chain HVR-H3, aLAG3(0411)
GLTDDTLYGSDY

SEQ ID NO: 33 - protein, 11 aa, Artificial Sequence
  light chain HVR-L1, aLAG3(0411)
RASQSIVSYLN

SEQ ID NO: 34 - protein, 7 aa, Artificial Sequence
  light chain HVR-L2, aLAG3(0411)
ASSSLQS

SEQ ID NO: 35 - protein, 9 aa, Artificial Sequence
  light chain HVR-L3, aLAG3(0411)
QQTYSTPLT

SEQ ID NO: 36 - protein, 121 aa, Artificial Sequence
  heavy chain variable domain VH, aLAG3(0411)
EVHLLESGGGLVQPGGSLRLSCAASGFIVDDYTMNWVRQAPGKGLEWVSVISWDGGATYYADSVKGRFTISRDDFKNTLYLQMNSLRAEDTAVYYCAKGLTDDTLYGSDYWGQGTLVTVSS

SEQ ID NO: 37 - protein, 107 aa, Artificial Sequence
  light chain variable domain VL, aLAG3(0411)
DIQMTQSPSSLSASVGDRVTITCRASQSIVSYLNWYQQKPGKAPKLLIYASSSLQSGVPSRFSGSGSGTDFTLTISSLQPEDFATYYCQQTYSTPLTFGGGTKVEIK

SEQ ID NO: 38 - protein, 5 aa, Artificial Sequence
  heavy chain HVR-H1, aLAG3(0417)
DYAMS

SEQ ID NO: 39 - protein, 17 aa, Artificial Sequence
  heavy chain HVR-H2, aLAG3(0417)
GIDNSGYYTYYTDSVKG

SEQ ID NO: 40 - protein, 13 aa, Artificial Sequence
  heavy chain HVR-H3, aLAG3(0417)
THSGLIVNDAFDI

SEQ ID NO: 41 - protein, 11 aa, Artificial Sequence
  light chain HVR-L1, aLAG3(0417)
RASQSISSYLN

SEQ ID NO: 42 - protein, 7 aa, Artificial Sequence
  light chain HVR-L2, aLAG3(0417)
AASSLQS

SEQ ID NO: 43 - protein, 9 aa, Artificial Sequence
  light chain HVR-L3, aLAG3(0417)
QQTYSTPLT

SEQ ID NO: 44 - protein, 122 aa, Artificial Sequence
  heavy chain variable domain VH, aLAG3(0417)
EVQLVESGGGLVQPGGSLRLACAASGFTFSDYAMSWVRQAPGKGLEWVSGIDNSGYYTYYTDSVKGRFTISRDDVKNTLYLQMNSLRAEDTAVYLCTKTHSGLIVNDAFDIWGQGTMVTVSS

SEQ ID NO: 45 - protein, 107 aa, Artificial Sequence
  light chain variable domain VL, aLAG3(0417)
DIQMTQSPSSLSASVGDRVTITCRASQSISSYLNWYQQKPGKAPKLLIYAASSLQSGVPSRFSGSGSGTDFTLTISSLQPEDFATYYCQQTYSTPLTFGGGTKVEIK

SEQ ID NO: 46 - protein, 5 aa, Artificial Sequence
  heavy chain HVR-H1, aLAG3(0416)
DYAMS

SEQ ID NO: 47 - protein, 17 aa, Artificial Sequence
  heavy chain HVR-H2, aLAG3(0416)
GIDNSGYYTYYTDSVKG

SEQ ID NO: 48 - protein, 13 aa, Artificial Sequence
  heavy chain HVR-H3, aLAG3(0416)
THSGLIVNDAFDI

SEQ ID NO: 49 - protein, 11 aa, Artificial Sequence
  light chain HVR-L1, aLAG3(0416)
RASQSISSYLN

SEQ ID NO: 50 - protein, 7 aa, Artificial Sequence
  light chain HVR-L2, aLAG3(0416)
DASSLES

SEQ ID NO: 51 - protein, 9 aa, Artificial Sequence
  light chain HVR-L3, aLAG3(0416)
QQSYSTPLT

SEQ ID NO: 52 - protein, 122 aa, Artificial Sequence; identical to SEQ ID NO: 44
  heavy chain variable domain VH, aLAG3(0416)

SEQ ID NO: 53 - protein, 107 aa, Artificial Sequence
  light chain variable domain VL, aLAG3(0416)
DIQLTQSPSSLSASVGDRVTITCRASQSISSYLNWYQQKPGKAPKLLIYDASSLESGVPSRFSGSGSGTDATLTISSLQPEDFATYYCQQSYSTPLTFGGGTKVEIK

SEQ ID NO: 54 - protein, 120 aa, Artificial Sequence
  heavy chain variable domain VH, BMS-986016
QVQLQQWGAGLLKPSETLSLTCAVYGGSFSDYYWNWIRQPPGKGLEWIGEINHRGSTNSNPSLKSRVTLSLDTSKNQFSLKLRSVTAADTAVYYCAFGYSDYEYNWFDPWGQGTLVTVSS

SEQ ID NO: 55 - protein, 107 aa, Artificial Sequence
  light chain variable domain VL BMS-986016
EIVLTQSPATLSLSPGERATLSCRASQSISSYLAWYQQKPGQAPRLLIYDASNRATGIPARFSGSGSGTDFTLTISSLEPEDFAVYYCQQRSNWPLTFGQGTNLEIK

SEQ ID NO: 56 - protein, 5 aa, Artificial Sequence
  heavy chain HVR-H1, MDX25F7 (25F7)
DYYWN

SEQ ID NO: 57 - protein, 16 aa, Artificial Sequence
  heavy chain HVR-H2, MDX25F7 (25F7)
EINHNGNTNSNPSLKS

SEQ ID NO: 58 - protein, 10 aa, Artificial Sequence
  heavy chain HVR-H3, MDX25F7 (25F7)
GYSDYEYNWF

SEQ ID NO: 59 - protein, 11 aa, Artificial Sequence
  light chain HVR-L1, MDX25F7 (25F7)
RASQSISSYLA

SEQ ID NO: 60 - protein, 7 aa, Artificial Sequence
  light chain HVR-L2, MDX25F7 (25F7)
DASNRAT

SEQ ID NO: 61 - protein, 9 aa, Artificial Sequence
  light chain HVR-L3, MDX25F7 (25F7)
QQRSNWPLT

SEQ ID NO: 62 - protein, 120 aa, Artificial Sequence
  heavy chain variable domain VH, MDX25F7 (25F7)
QVQLQQWGAGLLKPSETLSLTCAVYGGSFSDYYWNWIRQPPGKGLEWIGEINHNGNTNSNPSLKSRVTLSLDTSKNQFSLKLRSVTAADTAVYYCAFGYSDYEYNWFDPWGQGTLVTVSS

SEQ ID NO: 63 - protein, 107 aa, Artificial Sequence; identical to SEQ ID NO: 55
  light chain variable domain VL, MDX25F7 (25F7)

SEQ ID NO: 64 - protein, 125 aa, Artificial Sequence
  heavy chain variable domain VH, humanized BAP050 (LAG525)
QIQLVQSGPELKKPGETVKISCKASGFTLTNYGMNWVRQTPGKGLKWMGWINTDTGEPTYADDFKGRFAFSLETSASTASLQINNLKNADTATYFCARNPPYYYGTNNAEAMDYWGQGTTVTVSS

SEQ ID NO: 65 - protein, 107 aa, Artificial Sequence
  light chain variable domain VL, humanized BAP050 (LAG525)
DIQMTQTTSSLSASLGDRVTISCSSSQDISNYLMWYQQKPDGTVKVLIYYTSTLHLGVPSRFSGSGSGTDYSLTISNLELEDIATYYCQQYYNLPWTFGQGTKVEIK

SEQ ID NO: 66 - protein, 122 aa, Artificial Sequence
  heavy chain variable domain VH, MDX26H10 (26H10)
QVQLVESGGGVVQPGRSLRLSCAASGFTFSSYGMHWVRQAPGKGLEWVAVIWYDGSNKYYADSVKGRFTISRDNSKNTLYLQMNSLRAEDTAVYYCAREWAVASWDYGMDVWGQGTTVTVSS

SEQ ID NO: 67 - protein, 108 aa, Artificial Sequence
  light chain variable domain VL, MDX26H10 (26H10)
EIVLTQSPGTLSLSPGERATLSCRASQSVSSSYLAWYQQKPGQAPRLLIYGASSRATGIPDRFSGSGSGTDFTLTISRLEPEDFAVYYCQQYGSSPFTFGPGTKVDIK

SEQ ID NO: 68 - protein, 107 aa, Artificial Sequence [sequence omitted]

SEQ ID NO: 69 - protein, 105 aa, Artificial Sequence
  human lambda light chain constant region
QPKAAPSVTLFPPSSEELQANKATLVCLISDFYPGAVTVAWKADSSPVKAGVETTTPSKQSNNKYAASSYLSLTPEQWKSHRSYSCQVTHEGSTVEKTVAPTECS

SEQ ID NO: 70 - protein, 329 aa, Artificial Sequence
  human heavy chain constant region derived from IgG1
ASTKGPSVFPLAPSSKSTSGGTAALGCLVKDYFPEPVTVSWNSGALTSGVHTFPAVLQSSGLYSLSSVVTVPSSSLGTQTYICNVNHKPSNTKVDKKVEPKSCDKTHTCPPCPAPELLGGPSVFLFPPKPKDTLMISRTPEVTCVVVDVSHEDPEVKFNWYVDGVEVHNAKTKPREEQYNSTYRVVSVLTVLHQDWLNGKEYKCKVSNKALPAPIEKTISKAKGQPREPQVYTLPPSRDELTKNQVSLTCLVKGFYPSDIAVEWESNGQPENNYKTTPPVLDSDGSFFLYSKLTVDKSRWQQGNVFSCSVMHEALHNHYTQKSLSLSPG

SEQ ID NO: 71 - protein, 329 aa, Artificial Sequence
  human heavy chain constant region derived from IgG1 with mutations L234A, L235A and P329G
ASTKGPSVFPLAPSSKSTSGGTAALGCLVKDYFPEPVTVSWNSGALTSGVHTFPAVLQSSGLYSLSSVVTVPSSSLGTQTYICNVNHKPSNTKVDKKVEPKSCDKTHTCPPCPAPEAAGGPSVFLFPPKPKDTLMISRTPEVTCVVVDVSHEDPEVKFNWYVDGVEVHNAKTKPREEQYNSTYRVVSVLTVLHQDWLNGKEYKCKVSNKALGAPIEKTISKAKGQPREPQVYTLPPSRDELTKNQVSLTCLVKGFYPSDIAVEWESNGQPENNYKTTPPVLDSDGSFFLYSKLTVDKSRWQQGNVFSCSVMHEALHNHYTQKSLSLSPG

SEQ ID NO: 72 - protein, 326 aa, Artificial Sequence
  human heavy chain constant region derived from IgG4
ASTKGPSVFPLAPCSRSTSESTAALGCLVKDYFPEPVTVSWNSGALTSGVHTFPAVLQSSGLYSLSSVVTVPSSSLGTKTYTCNVDHKPSNTKVDKRVESKYGPPCPSCPAPEFLGGPSVFLFPPKPKDTLMISRTPEVTCVVVDVSQEDPEVQFNWYVDGVEVHNAKTKPREEQFNSTYRVVSVLTVLHQDWLNGKEYKCKVSNKGLPSSIEKTISKAKGQPREPQVYTLPPSQEEMTKNQVSLTCLVKGFYPSDIAVEWESNGQPENNYKTTPPVLDSDGSFFLYSRLTVDKSRWQEGNVFSCSVMHEALHNHYTQKSLSLSLG

SEQ ID NO: 73 - protein, 497 aa, Homo sapiens
VPVVWAQEGAPAQLPCSPTIPLQDLSLLRRAGVTWQHQPDSGPPAAAPGHPLAPGPHPAAPSSWGPRPRRYTVLSVGPGGLRSGRLPLQPRVQLDERGRQRGDFSLWLRPARRADAGEYRAAVHLRDRALSCRLRLRLGQASMTASPPGSLRASDWVILNCSFSRPDRPASVHWFRNRGQGRVPVRESPHHHLAESFLFLPQVSPMDSGPWGCILTYRDGFNVSIMYNLTVLGLEPPTPLTVYAGAGSRVGLPCRLPAGVGTRSFLTAKWTPPGGGPDLLVTGDNGDFTLRLEDVSQAQAGTYTCHIHLQEQQLNATVTLAIITVTPKSFGSPGSLGKLLCEVTPVSGQERFVWSSLDTPSQRSFSGPWLEAQEAQLLSQPWQCQLYQGERLLGAAVYFTELSSPGAQRSGRAPGALPAGHLLLFLILGVLSLLLLVTGAFGFHLWRRQWRPRRFSALEQGIHPPQAQSKIEELEQEPEPEPEPEPEPEPEPEPEQL

SEQ ID NO: 74 - protein, 422 aa, Homo sapiens
VPVVWAQEGAPAQLPCSPTIPLQDLSLLRRAGVTWQHQPDSGPPAAAPGHPLAPGPHPAAPSSWGPRPRRYTVLSVGPGGLRSGRLPLQPRVQLDERGRQRGDFSLWLRPARRADAGEYRAAVHLRDRALSCRLRLRLGQASMTASPPGSLRASDWVILNCSFSRPDRPASVHWFRNRGQGRVPVRESPHHHLAESFLFLPQVSPMDSGPWGCILTYRDGFNVSIMYNLTVLGLEPPTPLTVYAGAGSRVGLPCRLPAGVGTRSFLTAKWTPPGGGPDLLVTGDNGDFTLRLEDVSQAQAGTYTCHIHLQEQQLNATVTLAIITVTPKSFGSPGSLGKLLCEVTPVSGQERFVWSSLDTPSQRSFSGPWLEAQEAQLLSQPWQCQLYQGERLLGAAVYFTELSSPGAQRSGRAPGALPAGHL

SEQ ID NO: 75 - protein, 6 aa, Homo sapiens
KIEELE

SEQ ID NO: 76 - DNA, 37 bp, Artificial Sequence
  primer rbHC.up
aagcttgccaccatggagactgggctgcgctggcttc

SEQ ID NO: 77 - DNA, 21 bp, Artificial Sequence
  primer rbHCf.do
ccattggtgagggtgcccgag

SEQ ID NO: 78 - DNA, 20 bp, Artificial Sequence
  primer BcPCR_FHLC_leader.fw
atggacatgagggtccccgc

SEQ ID NO: 79 - DNA, 24 bp, Artificial Sequence
  primer BcPCR_huCkappa.rev
gatttcaactgctcatcagatggc

SEQ ID NO: 80 - protein, 8 aa, Artificial Sequence
  heavy chain HVR-H1, PD1-0098
GYSITSDY

SEQ ID NO: 81 - protein, 3 aa, Artificial Sequence
  heavy chain HVR-H2, PD1-0098
YSG

SEQ ID NO: 82 - protein, 9 aa, Artificial Sequence
  heavy chain HVR-H3, PD1-0098
HGSAPWYFD

SEQ ID NO: 83 - protein, 12 aa, Artificial Sequence
  light chain HVR-L1, PD1-0098
SQNIVHSDGNTY

SEQ ID NO: 84 - protein, 3 aa, Artificial Sequence
  light chain HVR-L2, PD1-0098
KVS

SEQ ID NO: 85 - protein, 6 aa, Artificial Sequence
  light chain HVR-L3, PD1-0098
GSHFPL

SEQ ID NO: 86 - protein, 120 aa, Artificial Sequence
  heavy chain variable domain VH, PD1-0098
DVQLQESGPGLVKPSQSLSLTCTVTGYSITSDYAWNWIRQFPGDKLEWLGYITYSGFTNYNPSLKSRISISRDTSKNQFFLQLNSVATEDTATYYCARWHGSAPWYFDYWGRGTTLTVSS

SEQ ID NO: 87 - protein, 112 aa, Artificial Sequence
  light chain variable domain VL, PD1-0098
DVLMTQTPLSLPVSLGDQASISCRSSQNIVHSDGNTYLEWYLQKPGQSPNLLIYKVSRRFSGVPDRFSGSGSGTDFTLKISRVEAEDLGVYYCFQGSHFPLTFGAGTKLELK

SEQ ID NO: 88 - protein, 7 aa, Artificial Sequence
  heavy chain HVR-H1, PD1-0069
GYTFTDY

SEQ ID NO: 89 - protein, 3 aa, Artificial Sequence
  heavy chain HVR-H2, PD1-0069
YSG

SEQ ID NO: 90 - protein, 7 aa, Artificial Sequence
  heavy chain HVR-H3, PD1-0069
GITTGFA

SEQ ID NO: 91 - protein, 11 aa, Artificial Sequence
  light chain HVR-L1, PD1-0069
SKGVSTSSYSF

SEQ ID NO: 92 - protein, 3 aa, Artificial Sequence
  light chain HVR-L2, PD1-0069
YAS

SEQ ID NO: 93 - protein, 6 aa, Artificial Sequence
  light chain HVR-L3, PD1-0069
SREFPW

SEQ ID NO: 94 - protein, 118 aa, Artificial Sequence
  heavy chain variable domain VH, PD1-0069
QVQLQQSGPELVRPGVSVKISCKGSGYTFTDYAMHWVKQSHARTLEWIGVISTYSGDTNYNQKFKDKATMTVDKSSSTAYLELARMTSEDSAIYYCARLGITTGFAYWGQGTLVTVSA

SEQ ID NO: 95 - protein, 111 aa, Artificial Sequence
  light chain variable domain VL, PD1-0069
DIVLTQSPASLAVSLGQRATISCRASKGVSTSSYSFMHWYQQKPRQPPKLLIKYASYLESGVPARFSGSGSGTDFTLNIHPVEEEDAATYYCHHSREFPWTFGGGTKLEIK

SEQ ID NO: 96 - protein, 443 aa, Artificial Sequence
  heavy chain 1 of 1+1 PD1/LAG3 0799
DIVMTQSPDSLAVSLGERATINCKASESVDTSDNSFIHWYQQKPGQSPKLLIYRSSTLESGVPDRFSGSGSGTDFTLTISSLQAEDVAVYYCQQNYDVPWTFGQGTKVEIKSSASTKGPSVFPLAPSSKSTSGGTAALGCLVKDYFPEPVTVSWNSGALTSGVHTFPAVLQSSGLYSLSSVVTVPSSSLGTQTYICNVNHKPSNTKVDKKVEPKSCDKTHTCPPCPAPEAAGGPSVFLFPPKPKDTLMISRTPEVTCVVVDVSHEDPEVKFNWYVDGVEVHNAKTKPREEQYNSTYRVVSVLTVLHQDWLNGKEYKCKVSNKALGAPIEKTISKAKGQPREPQVYTLPPCRDELTKNQVSLWCLVKGFYPSDIAVEWESNGQPENNYKTTPPVLDSDGSFFLYSKLTVDKSRWQQGNVFSCSVMHEALHNHYTQKSLSLSPGK

SEQ ID NO: 97 - protein, 452 aa, Artificial Sequence
  heavy chain 2 of 1+1 PD1/LAG3 0799
EVQLVESGGGLVQPGGSLRLACAASGFTFSDYAMSWVRQAPGKGLEWVSGIDNSGYYTYYTDSVKGRFTISRDDVKNTLYLQMNSLRAEDTAVYLCTKTHSGLIVNDAFDIWGQGTMVTVSSASTKGPSVFPLAPSSKSTSGGTAALGCLVEDYFPEPVTVSWNSGALTSGVHTFPAVLQSSGLYSLSSVVTVPSSSLGTQTYICNVNHKPSNTKVDEKVEPKSCDKTHTCPPCPAPEAAGGPSVFLFPPKPKDTLMISRTPEVTCVVVDVSHEDPEVKFNWYVDGVEVHNAKTKPREEQYNSTYRVVSVLTVLHQDWLNGKEYKCKVSNKALGAPIEKTISKAKGQPREPQVCTLPPSRDELTKNQVSLSCAVKGFYPSDIAVEWESNGQPENNYKTTPPVLDSDGSFFLVSKLTVDKSRWQQGNVFSCSVMHEALHNHYTQKSLSLSPGK

SEQ ID NO: 98 - protein, 227 aa, Artificial Sequence
  light chain 1 of 1+1 PD1/LAG3 0799
EVQLLESGGGLVQPGGSLRLSCAASGFSFSSYTMSWVRQAPGKGLEWVATISGGGRDIYYPDSVKGRFTISRDNSKNTLYLQMNSLRAEDTAVYYCVLLTGRVYFALDSWGQGTLVTVSSASVAAPSVFIFPPSDEQLKSGTASVVCLLNNFYPREAKVQWKVDNALQSGNSQESVTEQDSKDSTYSLSSTLTLSKADYEKHKVYACEVTHQGLSSPVTKSFNRGEC

SEQ ID NO: 99 - protein, 214 aa, Artificial Sequence
  light chain 2 of 1+1 PD1/LAG3 0799
DIQLTQSPSSLSASVGDRVTITCRASQSISSYLNWYQQKPGKAPKLLIYDASSLESGVPSRFSGSGSGTDATLTISSLQPEDFATYYCQQSYSTPLTFGGGTKVEIKRTVAAPSVFIFPPSDRKLKSGTASVVCLLNNFYPREAKVQWKVDNALQSGNSQESVTEQDSKDSTYSLSSTLTLSKADYEKHKVYACEVTHQGLSSPVTKSFNRGEC

SEQ ID NO: 100 - protein, 451 aa, Artificial Sequence
  heavy chain 2 of 1+1 PD1/LAG3 0927
EVQLLESGGGLVQPGGSLRLSCAASGFIFDDYTMNWVRQAPGKGLEWVAVISWDGGGTYYTDSVKGRFTISRDDFKNTLYLQMNSLRAEDTAVYYCAKGLTDTTLYGSDYWGQGTLVTVSSASTKGPSVFPLAPSSKSTSGGTAALGCLVEDYFPEPVTVSWNSGALTSGVHTFPAVLQSSGLYSLSSVVTVPSSSLGTQTYICNVNHKPSNTKVDEKVEPKSCDKTHTCPPCPAPEAAGGPSVFLFPPKPKDTLMISRTPEVTCVVVDVSHEDPEVKFNWYVDGVEVHNAKTKPREEQYNSTYRVVSVLTVLHQDWLNGKEYKCKVSNKALGAPIEKTISKAKGQPREPQVCTLPPSRDELTKNQVSLSCAVKGFYPSDIAVEWESNGQPENNYKTTPPVLDSDGSFFLVSKLTVDKSRWQQGNVFSCSVMHEALHNHYTQKSLSLSPGK

SEQ ID NO: 101 - protein, 214 aa, Artificial Sequence
  light chain 2 of 1+1 PD1/LAG3 0927
DIQMTQSPSSLSASVGDRVTITCRASQSISSYLNWYQQKPGKAPKLLIYAASTLQSGVPSRFSGSGSGTDFTLTISSLQPEDFATYYCQQTYSSPLTFGGGTKVEIKRTVAAPSVFIFPPSDRKLKSGTASVVCLLNNFYPREAKVQWKVDNALQSGNSQESVTEQDSKDSTYSLSSTLTLSKADYEKHKVYACEVTHQGLSSPVTKSFNRGEC

SEQ ID NO: 102 - protein, 443 aa, Artificial Sequence
  heavy chain 1 of 1+1 PD1/LAG3 0222
DIVLTQSPASLAVSLGQRATISCRASKGVSTSSYSFMHWYQQKPRQPPKLLIKYASYLESGVPARFSGSGSGTDFTLNIHPVEEEDAATYYCHHSREFPWTFGGGTKLEIKSSASTKGPSVFPLAPSSKSTSGGTAALGCLVKDYFPEPVTVSWNSGALTSGVHTFPAVLQSSGLYSLSSVVTVPSSSLGTQTYICNVNHKPSNTKVDKKVEPKSCDKTHTCPPCPAPEAAGGPSVFLFPPKPKDTLMISRTPEVTCVVVDVSHEDPEVKFNWYVDGVEVHNAKTKPREEQYNSTYRVVSVLTVLHQDWLNGKEYKCKVSNKALGAPIEKTISKAKGQPREPQVYTLPPCRDELTKNQVSLWCLVKGFYPSDIAVEWESNGQPENNYKTTPPVLDSDGSFFLYSKLTVDKSRWQQGNVFSCSVMHEALHNHYTQKSLSLSPGK

SEQ ID NO: 103 - protein, 450 aa, Artificial Sequence
  heavy chain 2 of 1+1 PD1/LAG3 0222
QVQLQQWGAGLLKPSETLSLTCAVYGGSFSDYYWNWIRQPPGKGLEWIGEINHNGNTNSNPSLKSRVTLSLDTSKNQFSLKLRSVTAADTAVYYCAFGYSDYEYNWFDPWGQGTLVTVSSASTKGPSVFPLAPSSKSTSGGTAALGCLVEDYFPEPVTVSWNSGALTSGVHTFPAVLQSSGLYSLSSVVTVPSSSLGTQTYICNVNHKPSNTKVDEKVEPKSCDKTHTCPPCPAPEAAGGPSVFLFPPKPKDTLMISRTPEVTCVVVDVSHEDPEVKFNWYVDGVEVHNAKTKPREEQYNSTYRVVSVLTVLHQDWLNGKEYKCKVSNKALGAPIEKTISKAKGQPREPQVCTLPPSRDELTKNQVSLSCAVKGFYPSDIAVEWESNGQPENNYKTTPPVLDSDGSFFLVSKLTVDKSRWQQGNVFSCSVMHEALHNHYTQKSLSLSPGK

SEQ ID NO: 104 - protein, 225 aa, Artificial Sequence
  light chain 1 of 1+1 PD1/LAG3 0222
QVQLQQSGPELVRPGVSVKISCKGSGYTFTDYAMHWVKQSHARTLEWIGVISTYSGDTNYNQKFKDKATMTVDKSSSTAYLELARMTSEDSAIYYCARLGITTGFAYWGQGTLVTVSAASVAAPSVFIFPPSDEQLKSGTASVVCLLNNFYPREAKVQWKVDNALQSGNSQESVTEQDSKDSTYSLSSTLTLSKADYEKHKVYACEVTHQGLSSPVTKSFNRGEC

SEQ ID NO: 105 - protein, 214 aa, Artificial Sequence
  light chain 2 of 1+1 PD1/LAG3 0222
EIVLTQSPATLSLSPGERATLSCRASQSISSYLAWYQQKPGQAPRLLIYDASNRATGIPARFSGSGSGTDFTLTISSLEPEDFAVYYCQQRSNWPLTFGQGTNLEIKRTVAAPSVFIFPPSDRKLKSGTASVVCLLNNFYPREAKVQWKVDNALQSGNSQESVTEQDSKDSTYSLSSTLTLSKADYEKHKVYACEVTHQGLSSPVTKSFNRGEC

SEQ ID NO: 106 - protein, 444 aa, Artificial Sequence
  heavy chain 1 of 1+1 PD1/LAG3 0224
DVLMTQTPLSLPVSLGDQASISCRSSQNIVHSDGNTYLEWYLQKPGQSPNLLIYKVSRRFSGVPDRFSGSGSGTDFTLKISRVEAEDLGVYYCFQGSHFPLTFGAGTKLELKSSASTKGPSVFPLAPSSKSTSGGTAALGCLVKDYFPEPVTVSWNSGALTSGVHTFPAVLQSSGLYSLSSVVTVPSSSLGTQTYICNVNHKPSNTKVDKKVEPKSCDKTHTCPPCPAPEAAGGPSVFLFPPKPKDTLMISRTPEVTCVVVDVSHEDPEVKFNWYVDGVEVHNAKTKPREEQYNSTYRVVSVLTVLHQDWLNGKEYKCKVSNKALGAPIEKTISKAKGQPREPQVYTLPPCRDELTKNQVSLWCLVKGFYPSDIAVEWESNGQPENNYKTTPPVLDSDGSFFLYSKLTVDKSRWQQGNVFSCSVMHEALHNHYTQKSLSLSPGK

SEQ ID NO: 107 - protein, 227 aa, Artificial Sequence
  light chain 1 of 1+1 PD1/LAG3 0224
DVQLQESGPGLVKPSQSLSLTCTVTGYSITSDYAWNWIRQFPGDKLEWLGYITYSGFTNYNPSLKSRISISRDTSKNQFFLQLNSVATEDTATYYCARWHGSAPWYFDYWGRGTTLTVSSASVAAPSVFIFPPSDEQLKSGTASVVCLLNNFYPREAKVQWKVDNALQSGNSQESVTEQDSKDSTYSLSSTLTLSKADYEKHKVYACEVTHQGLSSPVTKSFNRGEC

SEQ ID NO: 108 - protein, 443 aa, Artificial Sequence
  aLAG3(0156) heavy chain (MDX25F7)
QVQLQQWGAGLLKPSETLSLTCAVYGGSFSDYYWNWIRQPPGKGLEWIGEINHNGNTNSNPSLKSRVTLSLDTSKNQFSLKLRSVTAADTAVYYCAFGYSDYEYNWFDPWGQGTLVTVSSGQPKAPSVFPLAPCCGDTPSSTVTLGCLVKGYLPEPVTVTWNSGTLTNGVRTFPSVRQSSGLYSLSSVVSVTSSSQPVTCNVAHPATNTKVDKTVAPSTCSKPTCPPPELLGGPSVFIFPPKPKDTLMISRTPEVTCVVVDVSQDDPEVQFTWYINNEQVRTARPPLREQQFNSTIRVVSTLPIAHQDWLRGKEFKCKVHNKALPAPIEKTISKARGQPLEPKVYTMGPPREELSSRSVSLTCMINGFYPSDISVEWEKNGKAEDNYKTTPAVLDSDGSYFLYNKLSVPTSEWQRGDVFTCSVMHEALHNHYTQKSISRSPGK

SEQ ID NO: 109 - protein, 214 aa, Artificial Sequence
  aLAG3(0156) light chain (MDX25F7)
EIVLTQSPATLSLSPGERATLSCRASQSISSYLAWYQQKPGQAPRLLIYDASNRATGIPARFSGSGSGTDFTLTISSLEPEDFAVYYCQQRSNWPLTFGQGTNLEIKRTVAAPSVFIFPPSDEQLKSGTASVVCLLNNFYPREAKVQWKVDNALQSGNSQESVTEQDSKDSTYSLSSTLTLSKADYEKHKVYACEVTHQGLSSPVTKSFNRGEC

SEQ ID NO: 110 - protein, 444 aa, Artificial Sequence
  aLAG3(0414) heavy chain
EVQLLESGGGLVQPGGSLRLSCAASGFIFDDYTMNWVRQAPGKGLEWVAVISWDGGGTYYTDSVKGRFTISRDDFKNTLYLQMNSLRAEDTAVYYCAKGLTDTTLYGSDYWGQGTLVTVSSGQPKAPSVFPLAPCCGDTPSSTVTLGCLVKGYLPEPVTVTWNSGTLTNGVRTFPSVRQSSGLYSLSSVVSVTSSSQPVTCNVAHPATNTKVDKTVAPSTCSKPTCPPPELLGGPSVFIFPPKPKDTLMISRTPEVTCVVVDVSQDDPEVQFTWYINNEQVRTARPPLREQQFNSTIRVVSTLPIAHQDWLRGKEFKCKVHNKALPAPIEKTISKARGQPLEPKVYTMGPPREELSSRSVSLTCMINGFYPSDISVEWEKNGKAEDNYKTTPAVLDSDGSYFLYNKLSVPTSEWQRGDVFTCSVMHEALHNHYTQKSISRSPGK

SEQ ID NO: 111 - protein, 214 aa, Artificial Sequence
  aLAG3(0414) light chain
DIQMTQSPSSLSASVGDRVTITCRASQSISSYLNWYQQKPGKAPKLLIYAASTLQSGVPSRFSGSGSGTDFTLTISSLQPEDFATYYCQQTYSSPLTFGGGTKVEIKGTVAAPSVFIFPPSDEQLKSGTASVVCLLNNFYPREAKVQWKVDNALQSGNSQESVTEQDSKDSTYSLSSTLTLSKADYEKHKVYACEVTHQGLSSPVTKSFNRGEC

SEQ ID NO: 112 - protein, 445 aa, Artificial Sequence
  aLAG3(0416) heavy chain
EVQLVESGGGLVQPGGSLRLACAASGFTFSDYAMSWVRQAPGKGLEWVSGIDNSGYYTYYTDSVKGRFTISRDDVKNTLYLQMNSLRAEDTAVYLCTKTHSGLIVNDAFDIWGQGTMVTVSSGQPKAPSVFPLAPCCGDTPSSTVTLGCLVKGYLPEPVTVTWNSGTLTNGVRTFPSVRQSSGLYSLSSVVSVTSSSQPVTCNVAHPATNTKVDKTVAPSTCSKPTCPPPELLGGPSVFIFPPKPKDTLMISRTPEVTCVVVDVSQDDPEVQFTWYINNEQVRTARPPLREQQFNSTIRVVSTLPIAHQDWLRGKEFKCKVHNKALPAPIEKTISKARGQPLEPKVYTMGPPREELSSRSVSLTCMINGFYPSDISVEWEKNGKAEDNYKTTPAVLDSDGSYFLYNKLSVPTSEWQRGDVFTCSVMHEALHNHYTQKSISRSPGK

SEQ ID NO: 113 - protein, 214 aa, Artificial Sequence
  aLAG3(0416) light chain
DIQLTQSPSSLSASVGDRVTITCRASQSISSYLNWYQQKPGKAPKLLIYDASSLESGVPSRFSGSGSGTDATLTISSLQPEDFATYYCQQSYSTPLTFGGGTKVEIKGTVAAPSVFIFPPSDEQLKSGTASVVCLLNNFYPREAKVQWKVDNALQSGNSQESVTEQDSKDSTYSLSSTLTLSKADYEKHKVYACEVTHQGLSSPVTKSFNRGEC

SEQ ID NO: 114 - protein, 695 aa, Artificial Sequence
  heavy chain of 2+2 PD1/LAG3 8970
EVQLLESGGGLVQPGGSLRLSCAASGFIFDDYTMNWVRQAPGKGLEWVAVISWDGGGTYYTDSVKGRFTISRDDFKNTLYLQMNSLRAEDTAVYYCAKGLTDTTLYGSDYWGQGTLVTVSSASTKGPSVFPLAPSSKSTSGGTAALGCLVEDYFPEPVTVSWNSGALTSGVHTFPAVLQSSGLYSLSSVVTVPSSSLGTQTYICNVNHKPSNTKVDEKVEPKSCDKTHTCPPCPAPEAAGGPSVFLFPPKPKDTLMISRTPEVTCVVVDVSHEDPEVKFNWYVDGVEVHNAKTKPREEQYNSTYRVVSVLTVLHQDWLNGKEYKCKVSNKALGAPIEKTISKAKGQPREPQVYTLPPSRDELTKNQVSLTCLVKGFYPSDIAVEWESNGQPENNYKTTPPVLDSDGSFFLYSKLTVDKSRWQQGNVFSCSVMHEALHNHYTQKSLSLSPGGGSGGGGSGGGGSGGGGSEVQLLESGGGLVQPGGSLRLSCAASGFSFSSYTMSWVRQAPGKGLEWVATISGGGRDIYYPDSVKGRFTISRDNSKNTLYLQMNSLRAEDTAVYYCVLLTGRVYFALDSWGQGTLVTVSSASVAAPSVFIFPPSDEQLKSGTASVVCLLNNFYPREAKVQWKVDNALQSGNSQESVTEQDSKDSTYSLSSTLTLSKADYEKHKVYACEVTHQGLSSPVTKSFNRGEC

SEQ ID NO: 115 - protein, 216 aa, Artificial Sequence
  light chain 1 of 2+2 PD1/LAG3 8970
DIVMTQSPDSLAVSLGERATINCKASESVDTSDNSFIHWYQQKPGQSPKLLIYRSSTLESGVPDRFSGSGSGTDFTLTISSLQAEDVAVYYCQQNYDVPWTFGQGTKVEIKSSASTKGPSVFPLAPSSKSTSGGTAALGCLVKDYFPEPVTVSWNSGALTSGVHTFPAVLQSSGLYSLSSVVTVPSSSLGTQTYICNVNHKPSNTKVDKKVEPKSC

SEQ ID NO: 116 - protein, 696 aa, Artificial Sequence
  heavy chain of 2+2 PD1/LAG3 8984
EVQLVESGGGLVQPGGSLRLACAASGFTFSDYAMSWVRQAPGKGLEWVSGIDNSGYYTYYTDSVKGRFTISRDDVKNTLYLQMNSLRAEDTAVYLCTKTHSGLIVNDAFDIWGQGTMVTVSSASTKGPSVFPLAPSSKSTSGGTAALGCLVEDYFPEPVTVSWNSGALTSGVHTFPAVLQSSGLYSLSSVVTVPSSSLGTQTYICNVNHKPSNTKVDEKVEPKSCDKTHTCPPCPAPEAAGGPSVFLFPPKPKDTLMISRTPEVTCVVVDVSHEDPEVKFNWYVDGVEVHNAKTKPREEQYNSTYRVVSVLTVLHQDWLNGKEYKCKVSNKALGAPIEKTISKAKGQPREPQVYTLPPSRDELTKNQVSLTCLVKGFYPSDIAVEWESNGQPENNYKTTPPVLDSDGSFFLYSKLTVDKSRWQQGNVFSCSVMHEALHNHYTQKSLSLSPGGGSGGGGSGGGGSGGGGSEVQLLESGGGLVQPGGSLRLSCAASGFSFSSYTMSWVRQAPGKGLEWVATISGGGRDIYYPDSVKGRFTISRDNSKNTLYLQMNSLRAEDTAVYYCVLLTGRVYFALDSWGQGTLVTVSSASVAAPSVFIFPPSDEQLKSGTASVVCLLNNFYPREAKVQWKVDNALQSGNSQESVTEQDSKDSTYSLSSTLTLSKADYEKHKVYACEVTHQGLSSPVTKSFNRGEC

SEQ ID NO: 117 - protein, 694 aa, Artificial Sequence
  heavy chain of 2+2 PD1/LAG3 9010
QVQLQQWGAGLLKPSETLSLTCAVYGGSFSDYYWNWIRQPPGKGLEWIGEINHNGNTNSNPSLKSRVTLSLDTSKNQFSLKLRSVTAADTAVYYCAFGYSDYEYNWFDPWGQGTLVTVSSASTKGPSVFPLAPSSKSTSGGTAALGCLVEDYFPEPVTVSWNSGALTSGVHTFPAVLQSSGLYSLSSVVTVPSSSLGTQTYICNVNHKPSNTKVDEKVEPKSCDKTHTCPPCPAPEAAGGPSVFLFPPKPKDTLMISRTPEVTCVVVDVSHEDPEVKFNWYVDGVEVHNAKTKPREEQYNSTYRVVSVLTVLHQDWLNGKEYKCKVSNKALGAPIEKTISKAKGQPREPQVYTLPPSRDELTKNQVSLTCLVKGFYPSDIAVEWESNGQPENNYKTTPPVLDSDGSFFLYSKLTVDKSRWQQGNVFSCSVMHEALHNHYTQKSLSLSPGGGSGGGGSGGGGSGGGGSEVQLLESGGGLVQPGGSLRLSCAASGFSFSSYTMSWVRQAPGKGLEWVATISGGGRDIYYPDSVKGRFTISRDNSKNTLYLQMNSLRAEDTAVYYCVLLTGRVYFALDSWGQGTLVTVSSASVAAPSVFIFPPSDEQLKSGTASVVCLLNNFYPREAKVQWKVDNALQSGNSQESVTEQDSKDSTYSLSSTLTLSKADYEKHKVYACEVTHQGLSSPVTKSFNRGEC

SEQ ID NO: 118 - protein, 695 aa, Artificial Sequence
  heavy chain 1of 2+1 PD1/LAG3 8310
EVQLLESGGGLVQPGGSLRLSCAASGFIFDDYTMNWVRQAPGKGLEWVAVISWDGGGTYYTDSVKGRFTISRDDFKNTLYLQMNSLRAEDTAVYYCAKGLTDTTLYGSDYWGQGTLVTVSSASTKGPSVFPLAPSSKSTSGGTAALGCLVEDYFPEPVTVSWNSGALTSGVHTFPAVLQSSGLYSLSSVVTVPSSSLGTQTYICNVNHKPSNTKVDEKVEPKSCDKTHTCPPCPAPEAAGGPSVFLFPPKPKDTLMISRTPEVTCVVVDVSHEDPEVKFNWYVDGVEVHNAKTKPREEQYNSTYRVVSVLTVLHQDWLNGKEYKCKVSNKALGAPIEKTISKAKGQPREPQVYTLPPCRDELTKNQVSLWCLVKGFYPSDIAVEWESNGQPENNYKTTPPVLDSDGSFFLYSKLTVDKSRWQQGNVFSCSVMHEALHNHYTQKSLSLSPGGGSGGGGSGGGGSGGGGSEVQLLESGGGLVQPGGSLRLSCAASGFSFSSYTMSWVRQAPGKGLEWVATISGGGRDIYYPDSVKGRFTISRDNSKNTLYLQMNSLRAEDTAVYYCVLLTGRVYFALDSWGQGTLVTVSSASVAAPSVFIFPPSDEQLKSGTASVVCLLNNFYPREAKVQWKVDNALQSGNSQESVTEQDSKDSTYSLSSTLTLSKADYEKHKVYACEVTHQGLSSPVTKSFNRGEC

SEQ ID NO: 119 - protein, 451 aa, Artificial Sequence; identical to SEQ ID NO: 100
  heavy chain 2 of 2+1 PD1/LAG3 8310

SEQ ID NO: 120 - protein, 696 aa, Artificial Sequence
  heavy chain 1of 2+1 PD1/LAG3 8311
EVQLVESGGGLVQPGGSLRLACAASGFTFSDYAMSWVRQAPGKGLEWVSGIDNSGYYTYYTDSVKGRFTISRDDVKNTLYLQMNSLRAEDTAVYLCTKTHSGLIVNDAFDIWGQGTMVTVSSASTKGPSVFPLAPSSKSTSGGTAALGCLVEDYFPEPVTVSWNSGALTSGVHTFPAVLQSSGLYSLSSVVTVPSSSLGTQTYICNVNHKPSNTKVDEKVEPKSCDKTHTCPPCPAPEAAGGPSVFLFPPKPKDTLMISRTPEVTCVVVDVSHEDPEVKFNWYVDGVEVHNAKTKPREEQYNSTYRVVSVLTVLHQDWLNGKEYKCKVSNKALGAPIEKTISKAKGQPREPQVYTLPPCRDELTKNQVSLWCLVKGFYPSDIAVEWESNGQPENNYKTTPPVLDSDGSFFLYSKLTVDKSRWQQGNVFSCSVMHEALHNHYTQKSLSLSPGGGSGGGGSGGGGSGGGGSEVQLLESGGGLVQPGGSLRLSCAASGFSFSSYTMSWVRQAPGKGLEWVATISGGGRDIYYPDSVKGRFTISRDNSKNTLYLQMNSLRAEDTAVYYCVLLTGRVYFALDSWGQGTLVTVSSASVAAPSVFIFPPSDEQLKSGTASVVCLLNNFYPREAKVQWKVDNALQSGNSQESVTEQDSKDSTYSLSSTLTLSKADYEKHKVYACEVTHQGLSSPVTKSFNRGEC

SEQ ID NO: 121 - protein, 452 aa, Artificial Sequence; identical to SEQ ID NO: 97
  heavy chain 2of 2+1 PD1/LAG3 8311

SEQ ID NO: 122 - protein, 694 aa, Artificial Sequence
  heavy chain 1of 2+1 PD1/LAG3 1252
QVQLQQWGAGLLKPSETLSLTCAVYGGSFSDYYWNWIRQPPGKGLEWIGEINHNGNTNSNPSLKSRVTLSLDTSKNQFSLKLRSVTAADTAVYYCAFGYSDYEYNWFDPWGQGTLVTVSSASTKGPSVFPLAPSSKSTSGGTAALGCLVEDYFPEPVTVSWNSGALTSGVHTFPAVLQSSGLYSLSSVVTVPSSSLGTQTYICNVNHKPSNTKVDEKVEPKSCDKTHTCPPCPAPEAAGGPSVFLFPPKPKDTLMISRTPEVTCVVVDVSHEDPEVKFNWYVDGVEVHNAKTKPREEQYNSTYRVVSVLTVLHQDWLNGKEYKCKVSNKALGAPIEKTISKAKGQPREPQVYTLPPCRDELTKNQVSLWCLVKGFYPSDIAVEWESNGQPENNYKTTPPVLDSDGSFFLYSKLTVDKSRWQQGNVFSCSVMHEALHNHYTQKSLSLSPGGGSGGGGSGGGGSGGGGSEVQLLESGGGLVQPGGSLRLSCAASGFSFSSYTMSWVRQAPGKGLEWVATISGGGRDIYYPDSVKGRFTISRDNSKNTLYLQMNSLRAEDTAVYYCVLLTGRVYFALDSWGQGTLVTVSSASVAAPSVFIFPPSDEQLKSGTASVVCLLNNFYPREAKVQWKVDNALQSGNSQESVTEQDSKDSTYSLSSTLTLSKADYEKHKVYACEVTHQGLSSPVTKSFNRGEC

SEQ ID NO: 123 - protein, 941 aa, Artificial Sequence
  heavy chain 1of 2+1 PD1/LAG3 8312
EVQLLESGGGLVQPGGSLRLSCAASGFIFDDYTMNWVRQAPGKGLEWVAVISWDGGGTYYTDSVKGRFTISRDDFKNTLYLQMNSLRAEDTAVYYCAKGLTDTTLYGSDYWGQGTLVTVSSASTKGPSVFPLAPSSKSTSGGTAALGCLVEDYFPEPVTVSWNSGALTSGVHTFPAVLQSSGLYSLSSVVTVPSSSLGTQTYICNVNHKPSNTKVDEKVEPKSCDKTHTCPPCPAPEAAGGPSVFLFPPKPKDTLMISRTPEVTCVVVDVSHEDPEVKFNWYVDGVEVHNAKTKPREEQYNSTYRVVSVLTVLHQDWLNGKEYKCKVSNKALGAPIEKTISKAKGQPREPQVYTLPPCRDELTKNQVSLWCLVKGFYPSDIAVEWESNGQPENNYKTTPPVLDSDGSFFLYSKLTVDKSRWQQGNVFSCSVMHEALHNHYTQKSLSLSPGGGGGSGGGGSGGGGSGGGGSDIVMTQSPDSLAVSLGERATINCKASESVDTSDNSFIHWYQQKPGQSPKLLIYRSSTLESGVPDRFSGSGSGTDFTLTISSLQAEDVAVYYCQQNYDVPWTFGQGTKVEIKRTVAAPSVFIFPPSDEQLKSGTASVVCLLNNFYPREAKVQWKVDNALQSGNSQESVTEQDSKDSTYSLSSTLTLSKADYEKHKVYACEVTHQGLSSPVTKSFNRGECGGGGSGGGGSGGGGSGGGGSGGGGSGGGGSEVQLLESGGGLVQPGGSLRLSCAASGFSFSSYTMSWVRQAPGKGLEWVATISGGGRDIYYPDSVKGRFTISRDNSKNTLYLQMNSLRAEDTAVYYCVLLTGRVYFALDSWGQGTLVTVSSASTKGPSVFPLAPSSKSTSGGTAALGCLVKDYFPEPVTVSWNSGALTSGVHTFPAVLQSSGLYSLSSVVTVPSSSLGTQTYICNVNHKPSNTKVDKKVEPKSC

SEQ ID NO: 124 - protein, 942 aa, Artificial Sequence
  heavy chain 1of 2+1 PD1/LAG3 8313
EVQLVESGGGLVQPGGSLRLACAASGFTFSDYAMSWVRQAPGKGLEWVSGIDNSGYYTYYTDSVKGRFTISRDDVKNTLYLQMNSLRAEDTAVYLCTKTHSGLIVNDAFDIWGQGTMVTVSSASTKGPSVFPLAPSSKSTSGGTAALGCLVEDYFPEPVTVSWNSGALTSGVHTFPAVLQSSGLYSLSSVVTVPSSSLGTQTYICNVNHKPSNTKVDEKVEPKSCDKTHTCPPCPAPEAAGGPSVFLFPPKPKDTLMISRTPEVTCVVVDVSHEDPEVKFNWYVDGVEVHNAKTKPREEQYNSTYRVVSVLTVLHQDWLNGKEYKCKVSNKALGAPIEKTISKAKGQPREPQVYTLPPCRDELTKNQVSLWCLVKGFYPSDIAVEWESNGQPENNYKTTPPVLDSDGSFFLYSKLTVDKSRWQQGNVFSCSVMHEALHNHYTQKSLSLSPGGGGGSGGGGSGGGGSGGGGSDIVMTQSPDSLAVSLGERATINCKASESVDTSDNSFIHWYQQKPGQSPKLLIYRSSTLESGVPDRFSGSGSGTDFTLTISSLQAEDVAVYYCQQNYDVPWTFGQGTKVEIKRTVAAPSVFIFPPSDEQLKSGTASVVCLLNNFYPREAKVQWKVDNALQSGNSQESVTEQDSKDSTYSLSSTLTLSKADYEKHKVYACEVTHQGLSSPVTKSFNRGECGGGGSGGGGSGGGGSGGGGSGGGGSGGGGSEVQLLESGGGLVQPGGSLRLSCAASGFSFSSYTMSWVRQAPGKGLEWVATISGGGRDIYYPDSVKGRFTISRDNSKNTLYLQMNSLRAEDTAVYYCVLLTGRVYFALDSWGQGTLVTVSSASTKGPSVFPLAPSSKSTSGGTAALGCLVKDYFPEPVTVSWNSGALTSGVHTFPAVLQSSGLYSLSSVVTVPSSSLGTQTYICNVNHKPSNTKVDKKVEPKSC

SEQ ID NO: 125 - protein, 940 aa, Artificial Sequence
  heavy chain 1of 2+1 PD1/LAG3 1088
QVQLQQWGAGLLKPSETLSLTCAVYGGSFSDYYWNWIRQPPGKGLEWIGEINHNGNTNSNPSLKSRVTLSLDTSKNQFSLKLRSVTAADTAVYYCAFGYSDYEYNWFDPWGQGTLVTVSSASTKGPSVFPLAPSSKSTSGGTAALGCLVEDYFPEPVTVSWNSGALTSGVHTFPAVLQSSGLYSLSSVVTVPSSSLGTQTYICNVNHKPSNTKVDEKVEPKSCDKTHTCPPCPAPEAAGGPSVFLFPPKPKDTLMISRTPEVTCVVVDVSHEDPEVKFNWYVDGVEVHNAKTKPREEQYNSTYRVVSVLTVLHQDWLNGKEYKCKVSNKALGAPIEKTISKAKGQPREPQVYTLPPCRDELTKNQVSLWCLVKGFYPSDIAVEWESNGQPENNYKTTPPVLDSDGSFFLYSKLTVDKSRWQQGNVFSCSVMHEALHNHYTQKSLSLSPGGGGGSGGGGSGGGGSGGGGSDIVMTQSPDSLAVSLGERATINCKASESVDTSDNSFIHWYQQKPGQSPKLLIYRSSTLESGVPDRFSGSGSGTDFTLTISSLQAEDVAVYYCQQNYDVPWTFGQGTKVEIKRTVAAPSVFIFPPSDEQLKSGTASVVCLLNNFYPREAKVQWKVDNALQSGNSQESVTEQDSKDSTYSLSSTLTLSKADYEKHKVYACEVTHQGLSSPVTKSFNRGECGGGGSGGGGSGGGGSGGGGSGGGGSGGGGSEVQLLESGGGLVQPGGSLRLSCAASGFSFSSYTMSWVRQAPGKGLEWVATISGGGRDIYYPDSVKGRFTISRDNSKNTLYLQMNSLRAEDTAVYYCVLLTGRVYFALDSWGQGTLVTVSSASTKGPSVFPLAPSSKSTSGGTAALGCLVKDYFPEPVTVSWNSGALTSGVHTFPAVLQSSGLYSLSSVVTVPSSSLGTQTYICNVNHKPSNTKVDKKVEPKSC

SEQ ID NO: 126 - protein, 589 aa, Artificial Sequence
  heavy chain 1of 2+1 PD1/LAG3 0918
QVQLQQWGAGLLKPSETLSLTCAVYGGSFSDYYWNWIRQPPGKGLEWIGEINHNGNTNSNPSLKSRVTLSLDTSKNQFSLKLRSVTAADTAVYYCAFGYSDYEYNWFDPWGQGTLVTVSSASTKGPSVFPLAPSSKSTSGGTAALGCLVKDYFPEPVTVSWNSGALTSGVHTFPAVLQSSGLYSLSSVVTVPSSSLGTQTYICNVNHKPSNTKVDKKVEPKSCDKTHTCPPCPAPEAAGGPSVFLFPPKPKDTLMISRTPEVTCVVVDVSHEDPEVKFNWYVDGVEVHNAKTKPREEQYNSTYRVVSVLTVLHQDWLNGKEYKCKVSNKALGAPIEKTISKAKGQPREPQVCTLPPSRDELTKNQVSLSCAVKGFYPSDIAVEWESNGQPENNYKTTPPVLDSDGSFFLVSKLTVDKSRWQQGNVFSCSVMHEALHNHYTQKSLSLSPGGGGGSGGGGSGGGGSGGGGSEVQLLESGGGLVQPGGSLRLSCAASGFSFSSYTMSWVRQAPGKGLEWVATISGGGRDIYYPDSVKGRFTISRDNSKNTLYLQMNSLRAEDTAVYYCVLLTGRVYFALDSWGQGTLVTVSS

SEQ ID NO: 127 - protein, 580 aa, Artificial Sequence
  heavy chain 2 of 2+1 PD1/LAG3 0918
QVQLQQWGAGLLKPSETLSLTCAVYGGSFSDYYWNWIRQPPGKGLEWIGEINHNGNTNSNPSLKSRVTLSLDTSKNQFSLKLRSVTAADTAVYYCAFGYSDYEYNWFDPWGQGTLVTVSSASTKGPSVFPLAPSSKSTSGGTAALGCLVKDYFPEPVTVSWNSGALTSGVHTFPAVLQSSGLYSLSSVVTVPSSSLGTQTYICNVNHKPSNTKVDKKVEPKSCDKTHTCPPCPAPEAAGGPSVFLFPPKPKDTLMISRTPEVTCVVVDVSHEDPEVKFNWYVDGVEVHNAKTKPREEQYNSTYRVVSVLTVLHQDWLNGKEYKCKVSNKALGAPIEKTISKAKGQPREPQVYTLPPCRDELTKNQVSLWCLVKGFYPSDIAVEWESNGQPENNYKTTPPVLDSDGSFFLYSKLTVDKSRWQQGNVFSCSVMHEALHNHYTQKSLSLSPGGGGGSGGGGSGGGGSGGGGSDIVMTQSPDSLAVSLGERATINCKASESVDTSDNSFIHWYQQKPGQSPKLLIYRSSTLESGVPDRFSGSGSGTDFTLTISSLQAEDVAVYYCQQNYDVPWTFGQGTKVEIK

SEQ ID NO: 128 - protein, 288 aa, Homo sapiens
MQIPQAPWPVVWAVLQLGWRPGWFLDSPDRPWNPPTFSPALLVVTEGDNATFTCSFSNTSESFVLNWYRMSPSNQTDKLAAFPEDRSQPGQDCRFRVTQLPNGRDFHMSVVRARRNDSGTYLCGAISLAPKAQIKESLRAELRVTERRAEVPTAHPSPSPRPAGQFQTLVVGVVGGLLGSLVLLVWVLAVICSRAARGTIGARRTGQPLKEDPSAVPVFSVDYGELDFQWREKTPEPPVPCVPEQTEYATIVFPSGMGTSSPARRGSADGPRSAQPLRPEDGHCSWPL

SEQ ID NO: 129 - protein, 5 aa, Artificial Sequence
  Peptide linker G4S
GGGGS

SEQ ID NO: 130 - protein, 10 aa, Artificial Sequence
  Peptide linker (G4S)2
GGGGSGGGGS

SEQ ID NO: 131 - protein, 10 aa, Artificial Sequence
  Peptide linker (SG4)2
SGGGGSGGGG

SEQ ID NO: 132 - protein, 14 aa, Artificial Sequence
  Peptide linker G4(SG4)2
GGGGSGGGGSGGGG

SEQ ID NO: 133 - protein, 10 aa, Artificial Sequence
  Peptide linker
GSPGSSSSGS

SEQ ID NO: 134 - protein, 15 aa, Artificial Sequence
  Peptide linker (G4S)3
GGGGSGGGGSGGGGS

SEQ ID NO: 135 - protein, 20 aa, Artificial Sequence
  Peptide linker (G4S)4
GGGGSGGGGSGGGGSGGGGS

SEQ ID NO: 136 - protein, 8 aa, Artificial Sequence
  Peptide linker
GSGSGSGS

SEQ ID NO: 137 - protein, 8 aa, Artificial Sequence
  Peptide linker
GSGSGNGS

SEQ ID NO: 138 - protein, 8 aa, Artificial Sequence
  Peptide linker
GGSGSGSG

SEQ ID NO: 139 - protein, 6 aa, Artificial Sequence
  Peptide linker
GGSGSG

SEQ ID NO: 140 - protein, 4 aa, Artificial Sequence
  Peptide linker
GGSG

SEQ ID NO: 141 - protein, 8 aa, Artificial Sequence
  Peptide linker
GGSGNGSG

SEQ ID NO: 142 - protein, 8 aa, Artificial Sequence
  Peptide linker
GGNGSGSG

SEQ ID NO: 143 - protein, 6 aa, Artificial Sequence
  Peptide linker
GGNGSG

SEQ ID NO: 144 - protein, 461 aa, Artificial Sequence
  heavy chain 2 of 1+1 PD1/LAG3 0725 (1+1 trans)
DKTHTCPPCPAPEAAGGPSVFLFPPKPKDTLMISRTPEVTCVVVDVSHEDPEVKFNWYVDGVEVHNAKTKPREEQYNSTYRVVSVLTVLHQDWLNGKEYKCKVSNKALGAPIEKTISKAKGQPREPQVCTLPPSRDELTKNQVSLSCAVKGFYPSDIAVEWESNGQPENNYKTTPPVLDSDGSFFLVSKLTVDKSRWQQGNVFSCSVMHEALHNHYTQKSLSLSPGKGGGGSGGGGSEVQLLESGGGLVQPGGSLRLSCAASGFIFDDYTMNWVRQAPGKGLEWVAVISWDGGGTYYTDSVKGRFTISRDDFKNTLYLQMNSLRAEDTAVYYCAKGLTDTTLYGSDYWGQGTLVTVSSASTKGPSVFPLAPSSKSTSGGTAALGCLVEDYFPEPVTVSWNSGALTSGVHTFPAVLQSSGLYSLSSVVTVPSSSLGTQTYICNVNHKPSNTKVDEKVEPKSC

SEQ ID NO: 145 - protein, 685 aa, Artificial Sequence
  heavy chain 2 of 2+1 PD1/LAG3 0750 (2+1 trans)
EVQLLESGGGLVQPGGSLRLSCAASGFIFDDYTMNWVRQAPGKGLEWVAVISWDGGGTYYTDSVKGRFTISRDDFKNTLYLQMNSLRAEDTAVYYCAKGLTDTTLYGSDYWGQGTLVTVSSASTKGPSVFPLAPSSKSTSGGTAALGCLVEDYFPEPVTVSWNSGALTSGVHTFPAVLQSSGLYSLSSVVTVPSSSLGTQTYICNVNHKPSNTKVDEKVEPKSCDKTHTCPPCPAPEAAGGPSVFLFPPKPKDTLMISRTPEVTCVVVDVSHEDPEVKFNWYVDGVEVHNAKTKPREEQYNSTYRVVSVLTVLHQDWLNGKEYKCKVSNKALGAPIEKTISKAKGQPREPQVCTLPPSRDELTKNQVSLSCAVKGFYPSDIAVEWESNGQPENNYKTTPPVLDSDGSFFLVSKLTVDKSRWQQGNVFSCSVMHEALHNHYTQKSLSLSPGKGGGGSGGGGSEVQLLESGGGLVQPGGSLRLSCAASGFIFDDYTMNWVRQAPGKGLEWVAVISWDGGGTYYTDSVKGRFTISRDDFKNTLYLQMNSLRAEDTAVYYCAKGLTDTTLYGSDYWGQGTLVTVSSASTKGPSVFPLAPSSKSTSGGTAALGCLVEDYFPEPVTVSWNSGALTSGVHTFPAVLQSSGLYSLSSVVTVPSSSLGTQTYICNVNHKPSNTKVDEKVEPKSC

SEQ ID NO: 146 - protein, 215 aa, Artificial Sequence
  Light chain CEA (CEA TCB)
DIQMTQSPSSLSASVGDRVTITCKASAAVGTYVAWYQQKPGKAPKLLIYSASYRKRGVPSRFSGSGSGTDFTLTISSLQPEDFATYYCHQYYTYPLFTFGQGTKLEIKRTVAAPSVFIFPPSDEQLKSGTASVVCLLNNFYPREAKVQWKVDNALQSGNSQESVTEQDSKDSTYSLSSTLTLSKADYEKHKVYACEVTHQGLSSPVTKSFNRGEC

SEQ ID NO: 147 - protein, 214 aa, Artificial Sequence
  Light chain CD3 (CEA TCB)
QAVVTQEPSLTVSPGGTVTLTCGSSTGAVTTSNYANWVQEKPGQAFRGLIGGTNKRAPGTPARFSGSLLGGKAALTLSGAQPEDEAEYYCALWYSNLWVFGGGTKLTVLSSASTKGPSVFPLAPSSKSTSGGTAALGCLVKDYFPEPVTVSWNSGALTSGVHTFPAVLQSSGLYSLSSVVTVPSSSLGTQTYICNVNHKPSNTKVDKKVEPKSC

SEQ ID NO: 148 - protein, 694 aa, Artificial Sequence
  CEA CD3 crossfab VHck fc knob P329GLALA (CEA TCB)
QVQLVQSGAEVKKPGASVKVSCKASGYTFTEFGMNWVRQAPGQGLEWMGWINTKTGEATYVEEFKGRVTFTTDTSTSTAYMELRSLRSDDTAVYYCARWDFAYYVEAMDYWGQGTTVTVSSASTKGPSVFPLAPSSKSTSGGTAALGCLVKDYFPEPVTVSWNSGALTSGVHTFPAVLQSSGLYSLSSVVTVPSSSLGTQTYICNVNHKPSNTKVDKKVEPKSCDGGGGSGGGGSEVQLLESGGGLVQPGGSLRLSCAASGFTFSTYAMNWVRQAPGKGLEWVSRIRSKYNNYATYYADSVKGRFTISRDDSKNTLYLQMNSLRAEDTAVYYCVRHGNFGNSYVSWFAYWGQGTLVTVSSASVAAPSVFIFPPSDEQLKSGTASVVCLLNNFYPREAKVQWKVDNALQSGNSQESVTEQDSKDSTYSLSSTLTLSKADYEKHKVYACEVTHQGLSSPVTKSFNRGECDKTHTCPPCPAPEAAGGPSVFLFPPKPKDTLMISRTPEVTCVVVDVSHEDPEVKFNWYVDGVEVHNAKTKPREEQYNSTYRVVSVLTVLHQDWLNGKEYKCKVSNKALGAPIEKTISKAKGQPREPQVYTLPPCRDELTKNQVSLWCLVKGFYPSDIAVEWESNGQPENNYKTTPPVLDSDGSFFLYSKLTVDKSRWQQGNVFSCSVMHEALHNHYTQKSLSLSPGK

SEQ ID NO: 149 - protein, 451 aa, Artificial Sequence
  CEA VHCH1 Fc hole P329GLALA (CEA TCB)
QVQLVQSGAEVKKPGASVKVSCKASGYTFTEFGMNWVRQAPGQGLEWMGWINTKTGEATYVEEFKGRVTFTTDTSTSTAYMELRSLRSDDTAVYYCARWDFAYYVEAMDYWGQGTTVTVSSASTKGPSVFPLAPSSKSTSGGTAALGCLVKDYFPEPVTVSWNSGALTSGVHTFPAVLQSSGLYSLSSVVTVPSSSLGTQTYICNVNHKPSNTKVDKKVEPKSCDKTHTCPPCPAPEAAGGPSVFLFPPKPKDTLMISRTPEVTCVVVDVSHEDPEVKFNWYVDGVEVHNAKTKPREEQYNSTYRVVSVLTVLHQDWLNGKEYKCKVSNKALGAPIEKTISKAKGQPREPQVCTLPPSRDELTKNQVSLSCAVKGFYPSDIAVEWESNGQPENNYKTTPPVLDSDGSFFLVSKLTVDKSRWQQGNVFSCSVMHEALHNHYTQKSLSLSPGK

SEQ ID NO: 150 - protein, 232 aa, Artificial Sequence
  CD3 VH-CL (CEACAM5 TCB)
EVQLLESGGGLVQPGGSLRLSCAASGFTFSTYAMNWVRQAPGKGLEWVSRIRSKYNNYATYYADSVKGRFTISRDDSKNTLYLQMNSLRAEDTAVYYCVRHGNFGNSYVSWFAYWGQGTLVTVSSASVAAPSVFIFPPSDEQLKSGTASVVCLLNNFYPREAKVQWKVDNALQSGNSQESVTEQDSKDSTYSLSSTLTLSKADYEKHKVYACEVTHQGLSSPVTKSFNRGEC

SEQ ID NO: 151 - protein, 449 aa, Artificial Sequence
  CEACAM5 VH-CH1(EE)-Fc (hole, P329G LALA)
QVQLVQSGAEVKKPGSSVKVSCKASGFNIKDTYMHWVRQAPGQGLEWMGRIDPANGNSKYVPKFQGRVTITADTSTSTAYMELSSLRSEDTAVYYCAPFGYYVSDYAMAYWGQGTLVTVSSASTKGPSVFPLAPSSKSTSGGTAALGCLVEDYFPEPVTVSWNSGALTSGVHTFPAVLQSSGLYSLSSVVTVPSSSLGTQTYICNVNHKPSNTKVDEKVEPKSCDKTHTCPPCPAPEAAGGPSVFLFPPKPKDTLMISRTPEVTCVVVDVSHEDPEVKFNWYVDGVEVHNAKTKPREEQYNSTYRVVSVLTVLHQDWLNGKEYKCKVSNKALGAPIEKTISKAKGQPREPQVCTLPPSRDELTKNQVSLSCAVKGFYPSDIAVEWESNGQPENNYKTTPPVLDSDGSFFLVSKLTVDKSRWQQGNVFSCSVMHEALHNHYTQKSLSLSP

SEQ ID NO: 152 - protein, 674 aa, Artificial Sequence
  CEACAM5 VH-CH1(EE)-CD3 VL-CH1-Fc (knob, P329G LALA)
QVQLVQSGAEVKKPGSSVKVSCKASGFNIKDTYMHWVRQAPGQGLEWMGRIDPANGNSKYVPKFQGRVTITADTSTSTAYMELSSLRSEDTAVYYCAPFGYYVSDYAMAYWGQGTLVTVSSASTKGPSVFPLAPSSKSTSGGTAALGCLVEDYFPEPVTVSWNSGALTSGVHTFPAVLQSSGLYSLSSVVTVPSSSLGTQTYICNVNHKPSNTKVDEKVEPKSCDGGGGSGGGGSQAVVTQEPSLTVSPGGTVTLTCGSSTGAVTTSNYANWVQEKPGQAFRGLIGGTNKRAPGTPARFSGSLLGGKAALTLSGAQPEDEAEYYCALWYSNLWVFGGGTKLTVLSSASTKGPSVFPLAPSSKSTSGGTAALGCLVKDYFPEPVTVSWNSGALTSGVHTFPAVLQSSGLYSLSSVVTVPSSSLGTQTYICNVNHKPSNTKVDKKVEPKSCDKTHTCPPCPAPEAAGGPSVFLFPPKPKDTLMISRTPEVTCVVVDVSHEDPEVKFNWYVDGVEVHNAKTKPREEQYNSTYRVVSVLTVLHQDWLNGKEYKCKVSNKALGAPIEKTISKAKGQPREPQVYTLPPCRDELTKNQVSLWCLVKGFYPSDIAVEWESNGQPENNYKTTPPVLDSDGSFFLYSKLTVDKSRWQQGNVFSCSVMHEALHNHYTQKSLSLSP

SEQ ID NO: 153 - protein, 218 aa, Artificial Sequence
  CEACAM5  VL-CL(RK)
EIVLTQSPATLSLSPGERATLSCRAGESVDIFGVGFLHWYQQKPGQAPRLLIYRASNRATGIPARFSGSGSGTDFTLTISSLEPEDFAVYYCQQTNEDPYTFGQGTKLEIKRTVAAPSVFIFPPSDRKLKSGTASVVCLLNNFYPREAKVQWKVDNALQSGNSQESVTEQDSKDSTYSLSSTLTLSKADYEKHKVYACEVTHQGLSSPVTKSFNRGEC

SEQ ID NO: 154 - protein, 5 aa, Artificial Sequence
  CEA-HCDR1
EFGMN

SEQ ID NO: 155 - protein, 17 aa, Artificial Sequence
  CEA-HCDR2
WINTKTGEATYVEEFKG

SEQ ID NO: 156 - protein, 12 aa, Artificial Sequence
  CEA-HCDR3
WDFAYYVEAMDY

SEQ ID NO: 157 - protein, 11 aa, Artificial Sequence
  CEA-LCDR1
KASAAVGTYVA

SEQ ID NO: 158 - protein, 7 aa, Artificial Sequence
  CEA-LCDR2
SASYRKR

SEQ ID NO: 159 - protein, 10 aa, Artificial Sequence
  CEA-LCDR3
HQYYTYPLFT

SEQ ID NO: 160 - protein, 121 aa, Artificial Sequence
  CEA VH
QVQLVQSGAEVKKPGASVKVSCKASGYTFTEFGMNWVRQAPGQGLEWMGWINTKTGEATYVEEFKGRVTFTTDTSTSTAYMELRSLRSDDTAVYYCARWDFAYYVEAMDYWGQGTTVTVSS

SEQ ID NO: 161 - protein, 108 aa, Artificial Sequence
  CEA VL
DIQMTQSPSSLSASVGDRVTITCKASAAVGTYVAWYQQKPGKAPKLLIYSASYRKRGVPSRFSGSGSGTDFTLTISSLQPEDFATYYCHQYYTYPLFTFGQGTKLEIK

SEQ ID NO: 162 - protein, 5 aa, Artificial Sequence
  CEA-HCDR1 (CEACAM5)
DTYMH

SEQ ID NO: 163 - protein, 17 aa, Artificial Sequence
  CEA-HCDR2 (CEACAM5)
RIDPANGNSKYVPKFQG

SEQ ID NO: 164 - protein, 12 aa, Artificial Sequence
  CEA-HCDR3 (CEACAM5)
FGYYVSDYAMAY

SEQ ID NO: 165 - protein, 15 aa, Artificial Sequence
  CEA-LCDR1 (CEACAM5)
RAGESVDIFGVGFLH

SEQ ID NO: 166 - protein, 7 aa, Artificial Sequence
  CEA-LCDR2 (CEACAM5)
RASNRAT

SEQ ID NO: 167 - protein, 9 aa, Artificial Sequence
  CEA-LCDR3 (CEACAM5)
QQTNEDPYT

SEQ ID NO: 168 - protein, 121 aa, Artificial Sequence
  CEA VH (CEACAM5)
QVQLVQSGAEVKKPGSSVKVSCKASGFNIKDTYMHWVRQAPGQGLEWMGRIDPANGNSKYVPKFQGRVTITADTSTSTAYMELSSLRSEDTAVYYCAPFGYYVSDYAMAYWGQGTLVTVSS

SEQ ID NO: 169 - protein, 111 aa, Artificial Sequence
  CEA VL (CEACAM5)
EIVLTQSPATLSLSPGERATLSCRAGESVDIFGVGFLHWYQQKPGQAPRLLIYRASNRATGIPARFSGSGSGTDFTLTISSLEPEDFAVYYCQQTNEDPYTFGQGTKLEIK